European Patent Application EP 4 293 039 A1, published December 20, 2023. Title: Novel IL-18 variant and use thereof. Applicant: Nagasaki University Foundation for Biomedical Research and Innovation at Kobe National Institutes for Quantum Science and Technology. The sequence listing filed with the application follows.

SEQUENCE LISTING (68 sequences)

SEQ ID NO: 1 - DNA, 973 bp, Homo sapiens
  CDS (221)..(802)
attctctccccagcttgctgagccctttgctcccctggcgactgcctggacagtcagcaaggaattgtctcccagtgcattttgccctcctggctgccaacgctggctgctaaagtggctgccacctgctgcagtctacacagcttcgggaagaggaaaggaacctcagaccttccagatcgcttcctctcgcaacaaactatttgtcgcaggaataaagatggctgctgaaccagtagaagacaattgcatcaactttgtggcaatgaaatttattgacaatacgctttactttatagctgaagatgatgaaaacctggaatccgattactttggcaagcttgaatctaaattatcagtcataagaaatttgaatgaccaagttctcttcattgaccaaggaaatcggcctctatttgaagatatgactgattctgactgtagagataatgcaccccggaccatatttattataagtatgtataaagatagccagcctagaggtatggctgtaactatctctgtgaagtgtgagaaaatttcaactctctcctgtgagaacaaaattatttcctttaaggaaatgaatcctcctgataacatcaaggatacaaaaagtgacatcatattctttcagagaagtgtcccaggacatgataataagatgcaatttgaatcttcatcatacgaaggatactttctagcttgtgaaaaagagagagacctttttaaactcattttgaaaaaagaggatgaattgggggatagatctataatgttcactgttcaaaacgaagactagctattaaaatttcatgccgggcgcagtggctcacgcctgtaatcccagccctttgggaggctgaggcgggcagatcgccagaggtcaggtgttcaagaccagcctgaccaacatggtgaaacctcatctctactaaaaatacaaaaaaaaaaaaaaaaaaaaaaaaaaaaa

SEQ ID NO: 2 - protein, 193 aa, Homo sapiens
MAAEPVEDNCINFVAMKFIDNTLYFIAEDDENLESDYFGKLESKLSVIRNLNDQVLFIDQGNRPLFEDMTDSDCRDNAPRTIFIISMYKDSQPRGMAVTISVKCEKISTLSCENKIISFKEMNPPDNIKDTKSDIIFFQRSVPGHDNKMQFESSSYEGYFLACEKERDLFKLILKKEDELGDRSIMFTVQNED

SEQ ID NO: 3 - protein, 157 aa, Homo sapiens
YFGKLESKLSVIRNLNDQVLFIDQGNRPLFEDMTDSDCRDNAPRTIFIISMYKDSQPRGMAVTISVKCEKISTLSCENKIISFKEMNPPDNIKDTKSDIIFFQRSVPGHDNKMQFESSSYEGYFLACEKERDLFKLILKKEDELGDRSIMFTVQNED

SEQ ID NO: 4 - DNA, 591 bp, Artificial Sequence
  NdeI-hProIL18-SalI
catatggctgctgaaccggttgaagacaactgcatcaacttcgttgctatgaaattcatcgacaacaccctgtacttcatcgctgaagacgacgaaaacctggaatctgactacttcggtaaactggaatctaaactgtctgttatccgtaacctgaacgaccaggttctgttcatcgaccagggtaaccgtccgctgttcgaagacatgaccgactctgactgccgtgacaacgctccgcgtaccatcttcatcatctctatgtacaaagactctcagccgcgtggtatggctgttaccatctctgttaaatgcgaaaaaatctctaccctgtcttgcgaaaacaaaatcatctctttcaaagaaatgaacccgccggacaacatcaaagacaccaaatctgacatcatcttcttccagcgttctgttccgggtcacgacaacaaaatgcagttcgaatcttcttcttacgaaggttacttcctggcttgcgaaaaagaacgtgacctgttcaaactgatcctgaaaaaagaagacgaactgggtgaccgttctatcatgttcaccgttcagaacgaagactaagtcgac

SEQ ID NO: 5 - protein, 157 aa, Artificial Sequence
  hIL-18-CS
YFGKLESKLSVIRNLNDQVLFIDQGNRPLFEDMTDSDSRDNAPRTIFIISMYKDSQPRGMAVTISVKSEKISTLSSENKIISFKEMNPPDNIKDTKSDIIFFQRSVPGHDNKMQFESSSYEGYFLASEKERDLFKLILKKEDELGDRSIMFTVQNED

SEQ ID NO: 6 - DNA, 480 bp, Artificial Sequence
  NdeI-hProIL18-CS-SalI
tacttcggtaaactggaatctaaactgtctgttatccgtaacctgaacgaccaggttctgttcatcgaccagggtaaccgtccgctgttcgaagacatgaccgactctgactctcgtgacaacgctccgcgtaccatcttcatcatctctatgtacaaagactctcagccgcgtggtatggctgttaccatctctgttaaatctgaaaaaatctctaccctgtcttctgaaaacaaaatcatctctttcaaagaaatgaacccgccggacaacatcaaagacaccaaatctgacatcatcttcttccagcgttctgttccgggtcacgacaacaaaatgcagttcgaatcttcttcttacgaaggttacttcctggcttctgaaaaagaacgtgacctgttcaaactgatcctgaaaaaagaagacgaactgggtgaccgttctatcatgttcaccgttcagaacgaagactaagtcgac

SEQ ID NO: 7 - protein, 157 aa, Artificial Sequence
  hIL-18-CSEK
YFGKLASKLSVIRNLNDQVLFIDQGNRPLFEDMTDSDSRDNAPRTIFIISMYADSQPRGMAVTISVKSEKISTLSSENKIISFKEMNPPDNIKDTKSDIIFFQRSVPGHDNKMQFESSSYEGYFLASEKERDLFKLILKKEDELGDRSIMFTVQNED

SEQ ID NO: 8 - DNA, 480 bp, Artificial Sequence
  NdeI-hProIL18-CSEK-SalI
tacttcggtaaactggcttctaaactgtctgttatccgtaacctgaacgaccaggttctgttcatcgaccagggtaaccgtccgctgttcgaagacatgaccgactctgactctcgtgacaacgctccgcgtaccatcttcatcatctctatgtacgctgactctcagccgcgtggtatggctgttaccatctctgttaaatctgaaaaaatctctaccctgtcttctgaaaacaaaatcatctctttcaaagaaatgaacccgccggacaacatcaaagacaccaaatctgacatcatcttcttccagcgttctgttccgggtcacgacaacaaaatgcagttcgaatcttcttcttacgaaggttacttcctggcttctgaaaaagaacgtgacctgttcaaactgatcctgaaaaaagaagacgaactgggtgaccgttctatcatgttcaccgttcagaacgaagactaagtcgac

SEQ ID NO: 9 - protein, 157 aa, Artificial Sequence
  hIL-18-CSEK-G3Y
YFYKLASKLSVIRNLNDQVLFIDQGNRPLFEDMTDSDSRDNAPRTIFIISMYADSQPRGMAVTISVKSEKISTLSSENKIISFKEMNPPDNIKDTKSDIIFFQRSVPGHDNKMQFESSSYEGYFLASEKERDLFKLILKKEDELGDRSIMFTVQNED

SEQ ID NO: 10 - DNA, 480 bp, Artificial Sequence
  NdeI-hProIL18-CSEK-G3Y-SalI
tacttctacaaactggcttctaaactgtctgttatccgtaacctgaacgaccaggttctgttcatcgaccagggtaaccgtccgctgttcgaagacatgaccgactctgactctcgtgacaacgctccgcgtaccatcttcatcatctctatgtacgctgactctcagccgcgtggtatggctgttaccatctctgttaaatctgaaaaaatctctaccctgtcttctgaaaacaaaatcatctctttcaaagaaatgaacccgccggacaacatcaaagacaccaaatctgacatcatcttcttccagcgttctgttccgggtcacgacaacaaaatgcagttcgaatcttcttcttacgaaggttacttcctggcttctgaaaaagaacgtgacctgttcaaactgatcctgaaaaaagaagacgaactgggtgaccgttctatcatgttcaccgttcagaacgaagactaagtcgac

SEQ ID NO: 11 - protein, 157 aa, Artificial Sequence
  hIL-18-CSEK-G3L
YFLKLASKLSVIRNLNDQVLFIDQGNRPLFEDMTDSDSRDNAPRTIFIISMYADSQPRGMAVTISVKSEKISTLSSENKIISFKEMNPPDNIKDTKSDIIFFQRSVPGHDNKMQFESSSYEGYFLASEKERDLFKLILKKEDELGDRSIMFTVQNED

SEQ ID NO: 12 - DNA, 480 bp, Artificial Sequence
  NdeI-hProIL18-CSEK-G3L-SalI
tacttcctgaaactggcttctaaactgtctgttatccgtaacctgaacgaccaggttctgttcatcgaccagggtaaccgtccgctgttcgaagacatgaccgactctgactctcgtgacaacgctccgcgtaccatcttcatcatctctatgtacgctgactctcagccgcgtggtatggctgttaccatctctgttaaatctgaaaaaatctctaccctgtcttctgaaaacaaaatcatctctttcaaagaaatgaacccgccggacaacatcaaagacaccaaatctgacatcatcttcttccagcgttctgttccgggtcacgacaacaaaatgcagttcgaatcttcttcttacgaaggttacttcctggcttctgaaaaagaacgtgacctgttcaaactgatcctgaaaaaagaagacgaactgggtgaccgttctatcatgttcaccgttcagaacgaagactaagtcgac

SEQ ID NO: 13 - protein, 157 aa, Artificial Sequence
  hIL-18-CSEK-A6W
YFGKLWSKLSVIRNLNDQVLFIDQGNRPLFEDMTDSDSRDNAPRTIFIISMYADSQPRGMAVTISVKSEKISTLSSENKIISFKEMNPPDNIKDTKSDIIFFQRSVPGHDNKMQFESSSYEGYFLASEKERDLFKLILKKEDELGDRSIMFTVQNED

SEQ ID NO: 14 - DNA, 480 bp, Artificial Sequence
  NdeI-hProIL18-CSEK-A6W-SalI
tacttcggtaaactgtggtctaaactgtctgttatccgtaacctgaacgaccaggttctgttcatcgaccagggtaaccgtccgctgttcgaagacatgaccgactctgactctcgtgacaacgctccgcgtaccatcttcatcatctctatgtacgctgactctcagccgcgtggtatggctgttaccatctctgttaaatctgaaaaaatctctaccctgtcttctgaaaacaaaatcatctctttcaaagaaatgaacccgccggacaacatcaaagacaccaaatctgacatcatcttcttccagcgttctgttccgggtcacgacaacaaaatgcagttcgaatcttcttcttacgaaggttacttcctggcttctgaaaaagaacgtgacctgttcaaactgatcctgaaaaaagaagacgaactgggtgaccgttctatcatgttcaccgttcagaacgaagactaagtcgac

SEQ ID NO: 15 - protein, 157 aa, Artificial Sequence
  hIL-18-CSEK-T34P
YFGKLASKLSVIRNLNDQVLFIDQGNRPLFEDMPDSDSRDNAPRTIFIISMYADSQPRGMAVTISVKSEKISTLSSENKIISFKEMNPPDNIKDTKSDIIFFQRSVPGHDNKMQFESSSYEGYFLASEKERDLFKLILKKEDELGDRSIMFTVQNED

SEQ ID NO: 16 - DNA, 480 bp, Artificial Sequence
  NdeI-hProIL18CSEK-T34P-SalI
tacttcggtaaactggcttctaaactgtctgttatccgtaacctgaacgaccaggttctgttcatcgaccagggtaaccgtccgctgttcgaagacatgccggactctgactctcgtgacaacgctccgcgtaccatcttcatcatctctatgtacgctgactctcagccgcgtggtatggctgttaccatctctgttaaatctgaaaaaatctctaccctgtcttctgaaaacaaaatcatctctttcaaagaaatgaacccgccggacaacatcaaagacaccaaatctgacatcatcttcttccagcgttctgttccgggtcacgacaacaaaatgcagttcgaatcttcttcttacgaaggttacttcctggcttctgaaaaagaacgtgacctgttcaaactgatcctgaaaaaagaagacgaactgggtgaccgttctatcatgttcaccgttcagaacgaagactaagtcgac

SEQ ID NO: 17 - protein, 157 aa, Artificial Sequence
  hIL-18-CSEK-C38M
YFGKLASKLSVIRNLNDQVLFIDQGNRPLFEDMTDSDMRDNAPRTIFIISMYADSQPRGMAVTISVKSEKISTLSSENKIISFKEMNPPDNIKDTKSDIIFFQRSVPGHDNKMQFESSSYEGYFLASEKERDLFKLILKKEDELGDRSIMFTVQNED

SEQ ID NO: 18 - DNA, 480 bp, Artificial Sequence
  NdeI-hProIL18CSEK-C38M-SalI
tacttcggtaaactggcttctaaactgtctgttatccgtaacctgaacgaccaggttctgttcatcgaccagggtaaccgtccgctgttcgaagacatgaccgactctgacatgcgtgacaacgctccgcgtaccatcttcatcatctctatgtacgctgactctcagccgcgtggtatggctgttaccatctctgttaaatctgaaaaaatctctaccctgtcttctgaaaacaaaatcatctctttcaaagaaatgaacccgccggacaacatcaaagacaccaaatctgacatcatcttcttccagcgttctgttccgggtcacgacaacaaaatgcagttcgaatcttcttcttacgaaggttacttcctggcttctgaaaaagaacgtgacctgttcaaactgatcctgaaaaaagaagacgaactgggtgaccgttctatcatgttcaccgttcagaacgaagactaagtcgac

SEQ ID NO: 19 - protein, 157 aa, Artificial Sequence
  hIL-18-CSEK-M51Y
YFGKLASKLSVIRNLNDQVLFIDQGNRPLFEDMTDSDSRDNAPRTIFIISYYADSQPRGMAVTISVKSEKISTLSSENKIISFKEMNPPDNIKDTKSDIIFFQRSVPGHDNKMQFESSSYEGYFLASEKERDLFKLILKKEDELGDRSIMFTVQNED

SEQ ID NO: 20 - DNA, 480 bp, Artificial Sequence
  NdeI-hProIL18CSEK-M51Y-SalI
tacttcggtaaactggcttctaaactgtctgttatccgtaacctgaacgaccaggttctgttcatcgaccagggtaaccgtccgctgttcgaagacatgaccgactctgactctcgtgacaacgctccgcgtaccatcttcatcatctcttactacgctgactctcagccgcgtggtatggctgttaccatctctgttaaatctgaaaaaatctctaccctgtcttctgaaaacaaaatcatctctttcaaagaaatgaacccgccggacaacatcaaagacaccaaatctgacatcatcttcttccagcgttctgttccgggtcacgacaacaaaatgcagttcgaatcttcttcttacgaaggttacttcctggcttctgaaaaagaacgtgacctgttcaaactgatcctgaaaaaagaagacgaactgggtgaccgttctatcatgttcaccgttcagaacgaagactaagtcgac

SEQ ID NO: 21 - protein, 157 aa, Artificial Sequence
  hIL-18-CSEK-S72Y
YFGKLASKLSVIRNLNDQVLFIDQGNRPLFEDMTDSDSRDNAPRTIFIISMYADSQPRGMAVTISVKSEKIYTLSSENKIISFKEMNPPDNIKDTKSDIIFFQRSVPGHDNKMQFESSSYEGYFLASEKERDLFKLILKKEDELGDRSIMFTVQNED

SEQ ID NO: 22 - DNA, 480 bp, Artificial Sequence
  NdeI-hProIL18CSEK-S72Y-SalI
tacttcggtaaactggcttctaaactgtctgttatccgtaacctgaacgaccaggttctgttcatcgaccagggtaaccgtccgctgttcgaagacatgaccgactctgactctcgtgacaacgctccgcgtaccatcttcatcatctctatgtacgctgactctcagccgcgtggtatggctgttaccatctctgttaaatctgaaaaaatctacaccctgtcttctgaaaacaaaatcatctctttcaaagaaatgaacccgccggacaacatcaaagacaccaaatctgacatcatcttcttccagcgttctgttccgggtcacgacaacaaaatgcagttcgaatcttcttcttacgaaggttacttcctggcttctgaaaaagaacgtgacctgttcaaactgatcctgaaaaaagaagacgaactgggtgaccgttctatcatgttcaccgttcagaacgaagactaagtcgac

SEQ ID NO: 23 - protein, 157 aa, Artificial Sequence
  hIL-18-CSEK-S72F
YFGKLASKLSVIRNLNDQVLFIDQGNRPLFEDMTDSDSRDNAPRTIFIISMYADSQPRGMAVTISVKSEKIFTLSSENKIISFKEMNPPDNIKDTKSDIIFFQRSVPGHDNKMQFESSSYEGYFLASEKERDLFKLILKKEDELGDRSIMFTVQNED

SEQ ID NO: 24 - DNA, 480 bp, Artificial Sequence
  NdeI-hProIL18CSEK-S72F-SalI
tacttcggtaaactggcttctaaactgtctgttatccgtaacctgaacgaccaggttctgttcatcgaccagggtaaccgtccgctgttcgaagacatgaccgactctgactctcgtgacaacgctccgcgtaccatcttcatcatctctatgtacgctgactctcagccgcgtggtatggctgttaccatctctgttaaatctgaaaaaatcttcaccctgtcttctgaaaacaaaatcatctctttcaaagaaatgaacccgccggacaacatcaaagacaccaaatctgacatcatcttcttccagcgttctgttccgggtcacgacaacaaaatgcagttcgaatcttcttcttacgaaggttacttcctggcttctgaaaaagaacgtgacctgttcaaactgatcctgaaaaaagaagacgaactgggtgaccgttctatcatgttcaccgttcagaacgaagactaagtcgac

SEQ ID NO: 25 - protein, 157 aa, Artificial Sequence
  hIL-18-CSEK-S72M
YFGKLASKLSVIRNLNDQVLFIDQGNRPLFEDMTDSDSRDNAPRTIFIISMYADSQPRGMAVTISVKSEKIMTLSSENKIISFKEMNPPDNIKDTKSDIIFFQRSVPGHDNKMQFESSSYEGYFLASEKERDLFKLILKKEDELGDRSIMFTVQNED

SEQ ID NO: 26 - DNA, 480 bp, Artificial Sequence
  NdeI-hProIL18CSEK-S72M-SalI
tacttcggtaaactggcttctaaactgtctgttatccgtaacctgaacgaccaggttctgttcatcgaccagggtaaccgtccgctgttcgaagacatgaccgactctgactctcgtgacaacgctccgcgtaccatcttcatcatctctatgtacgctgactctcagccgcgtggtatggctgttaccatctctgttaaatctgaaaaaatcatgaccctgtcttctgaaaacaaaatcatctctttcaaagaaatgaacccgccggacaacatcaaagacaccaaatctgacatcatcttcttccagcgttctgttccgggtcacgacaacaaaatgcagttcgaatcttcttcttacgaaggttacttcctggcttctgaaaaagaacgtgacctgttcaaactgatcctgaaaaaagaagacgaactgggtgaccgttctatcatgttcaccgttcagaacgaagactaagtcgac

SEQ ID NO: 27 - protein, 157 aa, Artificial Sequence
  hIL-18-CSEK-S72L
YFGKLASKLSVIRNLNDQVLFIDQGNRPLFEDMTDSDSRDNAPRTIFIISMYADSQPRGMAVTISVKSEKILTLSSENKIISFKEMNPPDNIKDTKSDIIFFQRSVPGHDNKMQFESSSYEGYFLASEKERDLFKLILKKEDELGDRSIMFTVQNED

SEQ ID NO: 28 - DNA, 480 bp, Artificial Sequence
  NdeI-hProIL18CSEK-S72L-SalI
tacttcggtaaactggcttctaaactgtctgttatccgtaacctgaacgaccaggttctgttcatcgaccagggtaaccgtccgctgttcgaagacatgaccgactctgactctcgtgacaacgctccgcgtaccatcttcatcatctctatgtacgctgactctcagccgcgtggtatggctgttaccatctctgttaaatctgaaaaaatcctgaccctgtcttctgaaaacaaaatcatctctttcaaagaaatgaacccgccggacaacatcaaagacaccaaatctgacatcatcttcttccagcgttctgttccgggtcacgacaacaaaatgcagttcgaatcttcttcttacgaaggttacttcctggcttctgaaaaagaacgtgacctgttcaaactgatcctgaaaaaagaagacgaactgggtgaccgttctatcatgttcaccgttcagaacgaagactaagtcgac

SEQ ID NO: 29 - protein, 157 aa, Artificial Sequence
  hIL-18-CSEK-S72W
YFGKLASKLSVIRNLNDQVLFIDQGNRPLFEDMTDSDSRDNAPRTIFIISMYADSQPRGMAVTISVKSEKIWTLSSENKIISFKEMNPPDNIKDTKSDIIFFQRSVPGHDNKMQFESSSYEGYFLASEKERDLFKLILKKEDELGDRSIMFTVQNED

SEQ ID NO: 30 - DNA, 480 bp, Artificial Sequence
  NdeI-hProIL18CSEK-S72W-SalI
tacttcggtaaactggcttctaaactgtctgttatccgtaacctgaacgaccaggttctgttcatcgaccagggtaaccgtccgctgttcgaagacatgaccgactctgactctcgtgacaacgctccgcgtaccatcttcatcatctctatgtacgctgactctcagccgcgtggtatggctgttaccatctctgttaaatctgaaaaaatctggaccctgtcttctgaaaacaaaatcatctctttcaaagaaatgaacccgccggacaacatcaaagacaccaaatctgacatcatcttcttccagcgttctgttccgggtcacgacaacaaaatgcagttcgaatcttcttcttacgaaggttacttcctggcttctgaaaaagaacgtgacctgttcaaactgatcctgaaaaaagaagacgaactgggtgaccgttctatcatgttcaccgttcagaacgaagactaagtcgac

SEQ ID NO: 31 - protein, 157 aa, Artificial Sequence
  hIL-18-CSEK-K112W
YFGKLASKLSVIRNLNDQVLFIDQGNRPLFEDMTDSDSRDNAPRTIFIISMYADSQPRGMAVTISVKSEKISTLSSENKIISFKEMNPPDNIKDTKSDIIFFQRSVPGHDNWMQFESSSYEGYFLASEKERDLFKLILKKEDELGDRSIMFTVQNED

SEQ ID NO: 32 - DNA, 480 bp, Artificial Sequence
  NdeI-hProIL18CSEK-K112W-SalI
tacttcggtaaactggcttctaaactgtctgttatccgtaacctgaacgaccaggttctgttcatcgaccagggtaaccgtccgctgttcgaagacatgaccgactctgactctcgtgacaacgctccgcgtaccatcttcatcatctctatgtacgctgactctcagccgcgtggtatggctgttaccatctctgttaaatctgaaaaaatctctaccctgtcttctgaaaacaaaatcatctctttcaaagaaatgaacccgccggacaacatcaaagacaccaaatctgacatcatcttcttccagcgttctgttccgggtcacgacaactggatgcagttcgaatcttcttcttacgaaggttacttcctggcttctgaaaaagaacgtgacctgttcaaactgatcctgaaaaaagaagacgaactgggtgaccgttctatcatgttcaccgttcagaacgaagactaagtcgac

SEQ ID NO: 33 - protein, 157 aa, Artificial Sequence
  hIL-18-CSEK-K119V
YFGKLASKLSVIRNLNDQVLFIDQGNRPLFEDMTDSDSRDNAPRTIFIISMYADSQPRGMAVTISVKSEKISTLSSENKIISFKEMNPPDNIKDTKSDIIFFQRSVPGHDNKMQFESSVYEGYFLASEKERDLFKLILKKEDELGDRSIMFTVQNED

SEQ ID NO: 34 - DNA, 480 bp, Artificial Sequence
  NdeI-hProIL18CSEK-K119V-SalI
tacttcggtaaactggcttctaaactgtctgttatccgtaacctgaacgaccaggttctgttcatcgaccagggtaaccgtccgctgttcgaagacatgaccgactctgactctcgtgacaacgctccgcgtaccatcttcatcatctctatgtacgctgactctcagccgcgtggtatggctgttaccatctctgttaaatctgaaaaaatctctaccctgtcttctgaaaacaaaatcatctctttcaaagaaatgaacccgccggacaacatcaaagacaccaaatctgacatcatcttcttccagcgttctgttccgggtcacgacaacaaaatgcagttcgaatcttctgtttacgaaggttacttcctggcttctgaaaaagaacgtgacctgttcaaactgatcctgaaaaaagaagacgaactgggtgaccgttctatcatgttcaccgttcagaacgaagactaagtcgac

SEQ ID NO: 35 - protein, 157 aa, Artificial Sequence
  hIL-18-CSEK-G145N
YFGKLASKLSVIRNLNDQVLFIDQGNRPLFEDMTDSDSRDNAPRTIFIISMYADSQPRGMAVTISVKSEKISTLSSENKIISFKEMNPPDNIKDTKSDIIFFQRSVPGHDNKMQFESSSYEGYFLASEKERDLFKLILKKEDELNDRSIMFTVQNED

SEQ ID NO: 36 - DNA, 480 bp, Artificial Sequence
  NdeI-hProIL18CSEK-G145N-SalI
tacttcggtaaactggcttctaaactgtctgttatccgtaacctgaacgaccaggttctgttcatcgaccagggtaaccgtccgctgttcgaagacatgaccgactctgactctcgtgacaacgctccgcgtaccatcttcatcatctctatgtacgctgactctcagccgcgtggtatggctgttaccatctctgttaaatctgaaaaaatctctaccctgtcttctgaaaacaaaatcatctctttcaaagaaatgaacccgccggacaacatcaaagacaccaaatctgacatcatcttcttccagcgttctgttccgggtcacgacaacaaaatgcagttcgaatcttcttcttacgaaggttacttcctggcttctgaaaaagaacgtgacctgttcaaactgatcctgaaaaaagaagacgaactgaacgaccgttctatcatgttcaccgttcagaacgaagactaagtcgac

SEQ ID NO: 37 - protein, 157 aa, Artificial Sequence
  hIL-18-CSEK-S7/50C
YFGKLACKLSVIRNLNDQVLFIDQGNRPLFEDMTDSDSRDNAPRTIFIICMYADSQPRGMAVTISVKSEKISTLSSENKIISFKEMNPPDNIKDTKSDIIFFQRSVPGHDNKMQFESSSYEGYFLASEKERDLFKLILKKEDELGDRSIMFTVQNED

SEQ ID NO: 38 - DNA, 480 bp, Artificial Sequence
  NdeI-hProIL18CSEK-S7/50C-SalI
tacttcggtaaactggcttgcaaactgtctgttatccgtaacctgaacgaccaggttctgttcatcgaccagggtaaccgtccgctgttcgaagacatgaccgactctgactctcgtgacaacgctccgcgtaccatcttcatcatctgcatgtacgctgactctcagccgcgtggtatggctgttaccatctctgttaaatctgaaaaaatctctaccctgtcttctgaaaacaaaatcatctctttcaaagaaatgaacccgccggacaacatcaaagacaccaaatctgacatcatcttcttccagcgttctgttccgggtcacgacaacaaaatgcagttcgaatcttcttcttacgaaggttacttcctggcttctgaaaaagaacgtgacctgttcaaactgatcctgaaaaaagaagacgaactgggtgaccgttctatcatgttcaccgttcagaacgaagactaagtcgac

SEQ ID NO: 39 - protein, 273 aa, Homo sapiens
ALKLCPHEEFLRLCKERAEEIYPIKERNNRTRLALIICNTEFDHLPPRNGADFDITGMKELLEGLDYSVDVEENLTARDMESALRAFATRPEHKSSDSTFLVLMSHGILEGICGTVHDEKKPDVLLYDTIFQIFNNRNCLSLKDKPKVIIVQACRGANRGELWVRDSPASLEVASSQSSENLEEDAVYKTHVEKDFIAFCSSTPHNVSWRDSTMGSIFITQLITCFQKYSWCCHLEEVFRKVQQSFETPRAKAQMPTIERLSMTRYFYLFPGN

SEQ ID NO: 40 - protein, 377 aa, Artificial Sequence
  hCasp4-D315E
MAEGNHRKKPLKVLESLGKDFLTGVLDNLVEQNVLNWKEEEKKKYYDAKTEDKVRVMADSMQEKQRMAGQMLLQTFFNIDQISPNKKAHPNMEAGPPESGESTDALKLCPHEEFLRLCKERAEEIYPIKERNNRTRLALIICNTEFDHLPPRNGADFDITGMKELLEGLDYSVDVEENLTARDMESALRAFATRPEHKSSDSTFLVLMSHGILEGICGTVHDEKKPDVLLYDTIFQIFNNRNCLSLKDKPKVIIVQACRGANRGELWVRDSPASLEVASSQSSENLEEDAVYKTHVEKDFIAFCSSTPHNVSWRESTMGSIFITQLITCFQKYSWCCHLEEVFRKVQQSFETPRAKAQMPTIERLSMTRYFYLFPGN

SEQ ID NO: 41 - DNA, 825 bp, Artificial Sequence
  hCasp4-D315E DNA
atggctctgaaactgtgcccgcacgaagaattcctgcgtctgtgcaaagaacgtgctgaagaaatctacccgatcaaagaacgtaacaaccgtacccgtctggctctgatcatctgcaacaccgaattcgaccacctgccgccgcgtaacggtgctgacttcgacatcaccggtatgaaagaactgctggaaggtctggactactctgttgacgttgaagaaaacctgaccgctcgtgacatggaatctgctctgcgtgctttcgctacccgtccggaacacaaatcttctgactctaccttcctggttctgatgtctcacggtatcctggaaggtatctgcggtaccgttcacgacgaaaaaaaaccggacgttctgctgtacgacaccatcttccagatcttcaacaaccgtaactgcctgtctctgaaagacaaaccgaaagttatcatcgttcaggcttgccgtggtgctaaccgtggtgaactgtgggttcgtgactctccggcttctctggaagttgcttcttctcagtcttctgaaaacctggaagaagacgctgtttacaaaacccacgttgaaaaagacttcatcgctttctgctcttctaccccgcacaacgtttcttggcgtgaatctaccatgggttctatcttcatcacccagctgatcacctgcttccagaaatactcttggtgctgccacctggaagaagttttccgtaaagttcagcagtctttcgaaaccccgcgtgctaaagctcagatgccgaccatcgaacgtctgtctatgacccgttacttctacctgttcccgggtaactaa

SEQ ID NO: 42 - DNA, 834 bp, Artificial Sequence
  NdeI-hCasp4-D315E-SalI
catatggctctgaaactgtgcccgcacgaagaattcctgcgtctgtgcaaagaacgtgctgaagaaatctacccgatcaaagaacgtaacaaccgtacccgtctggctctgatcatctgcaacaccgaattcgaccacctgccgccgcgtaacggtgctgacttcgacatcaccggtatgaaagaactgctggaaggtctggactactctgttgacgttgaagaaaacctgaccgctcgtgacatggaatctgctctgcgtgctttcgctacccgtccggaacacaaatcttctgactctaccttcctggttctgatgtctcacggtatcctggaaggtatctgcggtaccgttcacgacgaaaaaaaaccggacgttctgctgtacgacaccatcttccagatcttcaacaaccgtaactgcctgtctctgaaagacaaaccgaaagttatcatcgttcaggcttgccgtggtgctaaccgtggtgaactgtgggttcgtgactctccggcttctctggaagttgcttcttctcagtcttctgaaaacctggaagaagacgctgtttacaaaacccacgttgaaaaagacttcatcgctttctgctcttctaccccgcacaacgtttcttggcgtgaatctaccatgggttctatcttcatcacccagctgatcacctgcttccagaaatactcttggtgctgccacctggaagaagttttccgtaaagttcagcagtctttcgaaaccccgcgtgctaaagctcagatgccgaccatcgaacgtctgtctatgacccgttacttctacctgttcccgggtaactaagtcgac

SEQ ID NO: 43 - protein, 192 aa, Mus musculus
MAAMSEDSCVNFKEMMFIDNTLYFIPEENGDLESDNFGRLHCTTAVIRNINDQVLFVDKRQPVFEDMTDIDQSASEPQTRLIIYMYKDSEVRGLAVTLSVKDSKMSTLSCKNKIISFEEMDPPENIDDIQSDLIFFQKRVPGHNKMEFESSLYEGHFLACQKEDDAFKLILKKKDENGDKSVMFTLTNLHQS

SEQ ID NO: 44 - protein, 157 aa, Mus musculus
NFGRLHCTTAVIRNINDQVLFVDKRQPVFEDMTDIDQSASEPQTRLIIYMYKDSEVRGLAVTLSVKDSKMSTLSCKNKIISFEEMDPPENIDDIQSDLIFFQKRVPGHNKMEFESSLYEGHFLACQKEDDAFKLILKKKDENGDKSVMFTLTNLHQS

SEQ ID NO: 45 - protein, 157 aa, Artificial Sequence
  hIL-18-CS-G3Y
YFYKLESKLSVIRNLNDQVLFIDQGNRPLFEDMTDSDSRDNAPRTIFIISMYKDSQPRGMAVTISVKSEKISTLSSENKIISFKEMNPPDNIKDTKSDIIFFQRSVPGHDNKMQFESSSYEGYFLASEKERDLFKLILKKEDELGDRSIMFTVQNED

SEQ ID NO: 46 - DNA, 480 bp, Artificial Sequence
  NdeI-hProIL18CS-G3Y-SalI
tacttctacaaactggaatctaaactgtctgttatccgtaacctgaacgaccaggttctgttcatcgaccagggtaaccgtccgctgttcgaagacatgaccgactctgactctcgtgacaacgctccgcgtaccatcttcatcatctctatgtacaaagactctcagccgcgtggtatggctgttaccatctctgttaaatctgaaaaaatctctaccctgtcttctgaaaacaaaatcatctctttcaaagaaatgaacccgccggacaacatcaaagacaccaaatctgacatcatcttcttccagcgttctgttccgggtcacgacaacaaaatgcagttcgaatcttcttcttacgaaggttacttcctggcttctgaaaaagaacgtgacctgttcaaactgatcctgaaaaaagaagacgaactgggtgaccgttctatcatgttcaccgttcagaacgaagactaagtcgac

SEQ ID NO: 47 - protein, 157 aa, Artificial Sequence
  hIL-18-CS-G3L
YFLKLESKLSVIRNLNDQVLFIDQGNRPLFEDMTDSDSRDNAPRTIFIISMYKDSQPRGMAVTISVKSEKISTLSSENKIISFKEMNPPDNIKDTKSDIIFFQRSVPGHDNKMQFESSSYEGYFLASEKERDLFKLILKKEDELGDRSIMFTVQNED

SEQ ID NO: 48 - DNA, 480 bp, Artificial Sequence
  NdeI-hProIL18CS-G3L-SalI
tacttcctgaaactggaatctaaactgtctgttatccgtaacctgaacgaccaggttctgttcatcgaccagggtaaccgtccgctgttcgaagacatgaccgactctgactctcgtgacaacgctccgcgtaccatcttcatcatctctatgtacaaagactctcagccgcgtggtatggctgttaccatctctgttaaatctgaaaaaatctctaccctgtcttctgaaaacaaaatcatctctttcaaagaaatgaacccgccggacaacatcaaagacaccaaatctgacatcatcttcttccagcgttctgttccgggtcacgacaacaaaatgcagttcgaatcttcttcttacgaaggttacttcctggcttctgaaaaagaacgtgacctgttcaaactgatcctgaaaaaagaagacgaactgggtgaccgttctatcatgttcaccgttcagaacgaagactaagtcgac

SEQ ID NO: 49 - protein, 157 aa, Artificial Sequence
  hIL-18-CS-C38M
YFGKLESKLSVIRNLNDQVLFIDQGNRPLFEDMTDSDMRDNAPRTIFIISMYKDSQPRGMAVTISVKSEKISTLSSENKIISFKEMNPPDNIKDTKSDIIFFQRSVPGHDNKMQFESSSYEGYFLASEKERDLFKLILKKEDELGDRSIMFTVQNED

SEQ ID NO: 50 - DNA, 480 bp, Artificial Sequence
  NdeI-hProIL18CS-C38M-SalI
tacttcggtaaactggaatctaaactgtctgttatccgtaacctgaacgaccaggttctgttcatcgaccagggtaaccgtccgctgttcgaagacatgaccgactctgacatgcgtgacaacgctccgcgtaccatcttcatcatctctatgtacaaagactctcagccgcgtggtatggctgttaccatctctgttaaatctgaaaaaatctctaccctgtcttctgaaaacaaaatcatctctttcaaagaaatgaacccgccggacaacatcaaagacaccaaatctgacatcatcttcttccagcgttctgttccgggtcacgacaacaaaatgcagttcgaatcttcttcttacgaaggttacttcctggcttctgaaaaagaacgtgacctgttcaaactgatcctgaaaaaagaagacgaactgggtgaccgttctatcatgttcaccgttcagaacgaagactaagtcgac

SEQ ID NO: 51 - protein, 157 aa, Artificial Sequence
  hIL-18-CS-S72Y
YFGKLESKLSVIRNLNDQVLFIDQGNRPLFEDMTDSDSRDNAPRTIFIISMYKDSQPRGMAVTISVKSEKIYTLSSENKIISFKEMNPPDNIKDTKSDIIFFQRSVPGHDNKMQFESSSYEGYFLASEKERDLFKLILKKEDELGDRSIMFTVQNED

SEQ ID NO: 52 - DNA, 480 bp, Artificial Sequence
  NdeI-hProIL18CS-S72Y-SalI
tacttcggtaaactggaatctaaactgtctgttatccgtaacctgaacgaccaggttctgttcatcgaccagggtaaccgtccgctgttcgaagacatgaccgactctgactctcgtgacaacgctccgcgtaccatcttcatcatctctatgtacaaagactctcagccgcgtggtatggctgttaccatctctgttaaatctgaaaaaatctacaccctgtcttctgaaaacaaaatcatctctttcaaagaaatgaacccgccggacaacatcaaagacaccaaatctgacatcatcttcttccagcgttctgttccgggtcacgacaacaaaatgcagttcgaatcttcttcttacgaaggttacttcctggcttctgaaaaagaacgtgacctgttcaaactgatcctgaaaaaagaagacgaactgggtgaccgttctatcatgttcaccgttcagaacgaagactaagtcgac

SEQ ID NO: 53 - protein, 157 aa, Artificial Sequence
  hIL-18-CS-S72F
YFGKLESKLSVIRNLNDQVLFIDQGNRPLFEDMTDSDSRDNAPRTIFIISMYKDSQPRGMAVTISVKSEKIFTLSSENKIISFKEMNPPDNIKDTKSDIIFFQRSVPGHDNKMQFESSSYEGYFLASEKERDLFKLILKKEDELGDRSIMFTVQNED

SEQ ID NO: 54 - DNA, 480 bp, Artificial Sequence
  NdeI-hProIL18CS-S72F-SalI
tacttcggtaaactggaatctaaactgtctgttatccgtaacctgaacgaccaggttctgttcatcgaccagggtaaccgtccgctgttcgaagacatgaccgactctgactctcgtgacaacgctccgcgtaccatcttcatcatctctatgtacaaagactctcagccgcgtggtatggctgttaccatctctgttaaatctgaaaaaatcttcaccctgtcttctgaaaacaaaatcatctctttcaaagaaatgaacccgccggacaacatcaaagacaccaaatctgacatcatcttcttccagcgttctgttccgggtcacgacaacaaaatgcagttcgaatcttcttcttacgaaggttacttcctggcttctgaaaaagaacgtgacctgttcaaactgatcctgaaaaaagaagacgaactgggtgaccgttctatcatgttcaccgttcagaacgaagactaagtcgac

SEQ ID NO: 55 - protein, 157 aa, Artificial Sequence
  hIL-18-CS-S72M
YFGKLESKLSVIRNLNDQVLFIDQGNRPLFEDMTDSDSRDNAPRTIFIISMYKDSQPRGMAVTISVKSEKIMTLSSENKIISFKEMNPPDNIKDTKSDIIFFQRSVPGHDNKMQFESSSYEGYFLASEKERDLFKLILKKEDELGDRSIMFTVQNED

SEQ ID NO: 56 - DNA, 480 bp, Artificial Sequence
  NdeI-hProIL18CS-S72M-SalI
tacttcggtaaactggaatctaaactgtctgttatccgtaacctgaacgaccaggttctgttcatcgaccagggtaaccgtccgctgttcgaagacatgaccgactctgactctcgtgacaacgctccgcgtaccatcttcatcatctctatgtacaaagactctcagccgcgtggtatggctgttaccatctctgttaaatctgaaaaaatcatgaccctgtcttctgaaaacaaaatcatctctttcaaagaaatgaacccgccggacaacatcaaagacaccaaatctgacatcatcttcttccagcgttctgttccgggtcacgacaacaaaatgcagttcgaatcttcttcttacgaaggttacttcctggcttctgaaaaagaacgtgacctgttcaaactgatcctgaaaaaagaagacgaactgggtgaccgttctatcatgttcaccgttcagaacgaagactaagtcgac

SEQ ID NO: 57 - protein, 157 aa, Artificial Sequence
  hIL-18-G3Y
YFYKLESKLSVIRNLNDQVLFIDQGNRPLFEDMTDSDCRDNAPRTIFIISMYKDSQPRGMAVTISVKCEKISTLSCENKIISFKEMNPPDNIKDTKSDIIFFQRSVPGHDNKMQFESSSYEGYFLACEKERDLFKLILKKEDELGDRSIMFTVQNED

SEQ ID NO: 58 - DNA, 480 bp, Artificial Sequence
  NdeI-hProIL18-G3Y-SalI
tacttctacaaactggaatctaaactgtctgttatccgtaacctgaacgaccaggttctgttcatcgaccagggtaaccgtccgctgttcgaagacatgaccgactctgactgccgtgacaacgctccgcgtaccatcttcatcatctctatgtacaaagactctcagccgcgtggtatggctgttaccatctctgttaaatgcgaaaaaatctctaccctgtcttgcgaaaacaaaatcatctctttcaaagaaatgaacccgccggacaacatcaaagacaccaaatctgacatcatcttcttccagcgttctgttccgggtcacgacaacaaaatgcagttcgaatcttcttcttacgaaggttacttcctggcttgcgaaaaagaacgtgacctgttcaaactgatcctgaaaaaagaagacgaactgggtgaccgttctatcatgttcaccgttcagaacgaagactaagtcgac

SEQ ID NO: 59 - protein, 157 aa, Artificial Sequence
  hIL-18-G3L
YFLKLESKLSVIRNLNDQVLFIDQGNRPLFEDMTDSDCRDNAPRTIFIISMYKDSQPRGMAVTISVKCEKISTLSCENKIISFKEMNPPDNIKDTKSDIIFFQRSVPGHDNKMQFESSSYEGYFLACEKERDLFKLILKKEDELGDRSIMFTVQNED

SEQ ID NO: 60 - DNA, 480 bp, Artificial Sequence
  NdeI-hProIL18-G3L-SalI
tacttcctgaaactggaatctaaactgtctgttatccgtaacctgaacgaccaggttctgttcatcgaccagggtaaccgtccgctgttcgaagacatgaccgactctgactgccgtgacaacgctccgcgtaccatcttcatcatctctatgtacaaagactctcagccgcgtggtatggctgttaccatctctgttaaatgcgaaaaaatctctaccctgtcttgcgaaaacaaaatcatctctttcaaagaaatgaacccgccggacaacatcaaagacaccaaatctgacatcatcttcttccagcgttctgttccgggtcacgacaacaaaatgcagttcgaatcttcttcttacgaaggttacttcctggcttgcgaaaaagaacgtgacctgttcaaactgatcctgaaaaaagaagacgaactgggtgaccgttctatcatgttcaccgttcagaacgaagactaagtcgac

SEQ ID NO: 61 - protein, 157 aa, Artificial Sequence
  hIL-18-C38M
YFGKLESKLSVIRNLNDQVLFIDQGNRPLFEDMTDSDMRDNAPRTIFIISMYKDSQPRGMAVTISVKCEKISTLSCENKIISFKEMNPPDNIKDTKSDIIFFQRSVPGHDNKMQFESSSYEGYFLACEKERDLFKLILKKEDELGDRSIMFTVQNED

SEQ ID NO: 62 - DNA, 480 bp, Artificial Sequence
  NdeI-hProIL18-C38M-SalI
tacttcggtaaactggaatctaaactgtctgttatccgtaacctgaacgaccaggttctgttcatcgaccagggtaaccgtccgctgttcgaagacatgaccgactctgacatgcgtgacaacgctccgcgtaccatcttcatcatctctatgtacaaagactctcagccgcgtggtatggctgttaccatctctgttaaatgcgaaaaaatctctaccctgtcttgcgaaaacaaaatcatctctttcaaagaaatgaacccgccggacaacatcaaagacaccaaatctgacatcatcttcttccagcgttctgttccgggtcacgacaacaaaatgcagttcgaatcttcttcttacgaaggttacttcctggcttgcgaaaaagaacgtgacctgttcaaactgatcctgaaaaaagaagacgaactgggtgaccgttctatcatgttcaccgttcagaacgaagactaagtcgac

SEQ ID NO: 63 - protein, 157 aa, Artificial Sequence
  hIL-18-S72Y
YFGKLESKLSVIRNLNDQVLFIDQGNRPLFEDMTDSDCRDNAPRTIFIISMYKDSQPRGMAVTISVKCEKIYTLSCENKIISFKEMNPPDNIKDTKSDIIFFQRSVPGHDNKMQFESSSYEGYFLACEKERDLFKLILKKEDELGDRSIMFTVQNED

SEQ ID NO: 64 - DNA, 480 bp, Artificial Sequence
  NdeI-hProIL18-S72Y-SalI
tacttcggtaaactggaatctaaactgtctgttatccgtaacctgaacgaccaggttctgttcatcgaccagggtaaccgtccgctgttcgaagacatgaccgactctgactgccgtgacaacgctccgcgtaccatcttcatcatctctatgtacaaagactctcagccgcgtggtatggctgttaccatctctgttaaatgcgaaaaaatctacaccctgtcttgcgaaaacaaaatcatctctttcaaagaaatgaacccgccggacaacatcaaagacaccaaatctgacatcatcttcttccagcgttctgttccgggtcacgacaacaaaatgcagttcgaatcttcttcttacgaaggttacttcctggcttgcgaaaaagaacgtgacctgttcaaactgatcctgaaaaaagaagacgaactgggtgaccgttctatcatgttcaccgttcagaacgaagactaagtcgac

SEQ ID NO: 65 - protein, 157 aa, Artificial Sequence
  hIL-18-S72F
YFGKLESKLSVIRNLNDQVLFIDQGNRPLFEDMTDSDCRDNAPRTIFIISMYKDSQPRGMAVTISVKCEKIFTLSCENKIISFKEMNPPDNIKDTKSDIIFFQRSVPGHDNKMQFESSSYEGYFLACEKERDLFKLILKKEDELGDRSIMFTVQNED

SEQ ID NO: 66 - DNA, 480 bp, Artificial Sequence
  NdeI-hProIL18-S72F-SalI
tacttcggtaaactggaatctaaactgtctgttatccgtaacctgaacgaccaggttctgttcatcgaccagggtaaccgtccgctgttcgaagacatgaccgactctgactgccgtgacaacgctccgcgtaccatcttcatcatctctatgtacaaagactctcagccgcgtggtatggctgttaccatctctgttaaatgcgaaaaaatcttcaccctgtcttgcgaaaacaaaatcatctctttcaaagaaatgaacccgccggacaacatcaaagacaccaaatctgacatcatcttcttccagcgttctgttccgggtcacgacaacaaaatgcagttcgaatcttcttcttacgaaggttacttcctggcttgcgaaaaagaacgtgacctgttcaaactgatcctgaaaaaagaagacgaactgggtgaccgttctatcatgttcaccgttcagaacgaagactaagtcgac

SEQ ID NO: 67 - protein, 157 aa, Artificial Sequence
  hIL-18-S72M
YFGKLESKLSVIRNLNDQVLFIDQGNRPLFEDMTDSDCRDNAPRTIFIISMYKDSQPRGMAVTISVKCEKIMTLSCENKIISFKEMNPPDNIKDTKSDIIFFQRSVPGHDNKMQFESSSYEGYFLACEKERDLFKLILKKEDELGDRSIMFTVQNED

SEQ ID NO: 68 - DNA, 480 bp, Artificial Sequence
  NdeI-hProIL18-S72M-SalI
tacttcggtaaactggaatctaaactgtctgttatccgtaacctgaacgaccaggttctgttcatcgaccagggtaaccgtccgctgttcgaagacatgaccgactctgactgccgtgacaacgctccgcgtaccatcttcatcatctctatgtacaaagactctcagccgcgtggtatggctgttaccatctctgttaaatgcgaaaaaatcatgaccctgtcttgcgaaaacaaaatcatctctttcaaagaaatgaacccgccggacaacatcaaagacaccaaatctgacatcatcttcttccagcgttctgttccgggtcacgacaacaaaatgcagttcgaatcttcttcttacgaaggttacttcctggcttgcgaaaaagaacgtgacctgttcaaactgatcctgaaaaaagaagacgaactgggtgaccgttctatcatgttcaccgttcagaacgaagactaagtcgac